European Patent Application EP 4 389 907 A1, published June 26, 2024. Title: Methods for the enzymatic treatment of whole stillage. Applicant: BASF SE. The sequence listing filed with the application follows.

SEQUENCE LISTING (1 sequence)

SEQ ID NO: 1 - protein, 317 aa, synthetic construct
  REGION 1..317: note = thermostable cellulase
MGVDPFERNKILGRGINIGNALEAPNEGDWGVVIKDEFFDIIKEAGFSHVRIPIRWSTHAQAFPPYKIEPSFFKRVDEVINGALKRGLAVVINIHHYEELMNDPEEHKERFLALWKQIADRYKDYPETLFFEILNEPHGNLTPEKWNELLEEALKVIRSIDKKHTVIIGTAEWGGISALEKLRVPKWEKNAIVTIHYYNPFEFTHQGAEWVPGSEKWLGRKWGSPDDQKHLIEEFNFIEEWSKKNKRPIYIGEFGAYRKADLESRIKWTSFVVREAEKRGWSWAYWEFCSGFGVYDPLRKQWNKDLLEALIGGDSIE